European Patent Application EP 4 450 650 A1, published October 23, 2024. Title: Method and system for risk assessment for poly-cystic ovarian syndrome (PCOS). Applicant: Tata Consultancy Services Limited. Application EP. The sequence listing filed with the application follows.

SEQUENCE LISTING (15 sequences)

SEQ ID NO: 1 - RNA, 1528 nt, Phocaeicola faecicola strain AGMB03916
  source 1..1528: mol_type = rRNA
acaatgaagagtttgatcctggctcaggatgaacgctagctacaggcttaacacatgcaagtcgaggggcagcgggattgaagcttgcttcaattgccggcgaccggcgcacgggtgagtaacacgtatccaaccttccgtttactcggggatagcctttcgaaagaaagattaatacccgatagtatggtgagattgcatgatagcaccattaaagattcatcggtaaacgatggggatgcgttccattaggtagtaggcggggtaacggcccacctagcctgcgatggataggggttctgagaggaaggtcccccacattggaactgagacacggtccaaactcctacgggaggcagcagtgaggaatattggtcaatgggcgagagcctgaaccagccaagtagcgtgaaggatgaaggtcctacggattgtaaacttcttttataagggaataaaacgctccacgtgtggagccttgtatgtaccttatgaataagcatcggctaactccgtgccagcagccgcggtaatacggaggatgcgagcgttatccggatttattgggtttaaagggagcgcagacgggatgttaagtcagctgtgaaagtttgcggctcaaccgtaaaattgcagttgatactggcgttcttgagtgcagttgaggtgtgcggaattcgtggtgtagcggtgaaatgcttagatatcacgaagaactccgattgcgaaggcagctcactaaactgtaactgacgttcatgctcgaaagtgtgggtatcaaacaggattagataccctggtagtccacacggtaaacgatggatactcgctgttggcgatatacggtcagcggccaagcgaaagcgttaagtatcccacctggggagtacgccggcaacggtgaaactcaaaggaattgacgggggcccgcacaagcggaggaacatgtggtttaattcgatgatacgcgaggaaccttacccgggcttaaattgcagaggaatgatctggaaacaggtcagtcttcggacttctgtgaaggtgctgcatggttgtcgtcagctcgtgccgtgaggtgtcggcttaagtgccataacgagcgcaacccttgtggtcagttactaacaggtaatgctgaggactctggccagactgccatcgtaagatgtgaggaaggcggggatgacgtcaaatcagcacggcccttacgtccggggctacacacgtgttacaatgggaggtacagaaggctgcgacccggcgacgggcagctaatcccaaaagcctctctcagttcggactggagtctgcaacccgactccacgaagctggattcgctagtaatcgcgcatcagccacggcgcggtgaatacgttcccgggccttgtacacaccgcccgtcaagccatgaaagccgggggtacctgaagtgcgtaaccgcaaggagcgtcctagggtaaaaccggtaattggggctaagtcgtaacaaggtagccgtaccggaaggtgcggctggaacacctccttt

SEQ ID NO: 2 - RNA, 1465 nt, Simonsiella muelleri ATCC 29453
  source 1..1465: mol_type = rRNA
attgaacgctggcggcatgctttacacatgcaagtcggacggcagcggggtagtgcttgcattactgccggcgagtggcgaacgggtgagtataatattggaacgtaccgagtaatgggggataactatccgaaaggatggctaataccgcatacgtcctgagggagaaagcgggggacaggcaactgcctcgcgttatttgagcggccaatatcggattagctagttggtggggtaaaggcttaccaaggcgacgatccgtagcgggtctgagaggatgatccgccacactgggactgagacacggcccagactcctacgggaggcagcagtggggaattttggacaatggggggaaccctgatccagccatgtcgcgtgtatgaagaaggccttagggttgtaaagtacttttgttagggaagaaaaggcatttgctaatatcagatgctgatgacggtacctaaagaataagcaccggctaactacgtgccagcagccgcggtaatacgtagggtgcgagcgttaatcggaattactgggcgtaaagcgagcgcagacggttacttaagcaagatgtgaaatccccgagctcaacttgggaactgcgttttgaactgggtagctagagtgtgtcagaggggggtagaattccacgtgtagcagtgaaatgcgtagagatgtggaggaataccgatggcgaaggcagccccctgggatagcactgacgttcatgctcgaaagcgtgggtagcaaacaggattagataccctggtagtccacgccctaaacgatgtcaattagctgttggggcactagatgccttagtagcgaagctaacgcgtgaaattgaccgcctggggagtacggtcgcaagattaaaactcaaaggaattgacggggacccgcacaagcggtggatgatgtggattaattcgatgcaacgcgaagaaccttacctggtcttgacatgtacggaatctctcagagacgggagagtgccttcgggagccgtaacacaggtgctgcatggctgtcgtcagctcgtgtcgtgagatgttgggttaagtcccgcaacgagcgcaacccttgtcattagttgccatcatttggttgggcactctaatgagactgccggtgacaaaccggaggaaggtggggatgacgtcaagtcctcatggcccttatgaccagggcttcacacgtcatacaatggtcggtacagagggtagccaagccgcgaggtggagccaatcccaaaaaaccgatcgtagtccggattgcactctgcaactcgagtgcatgaagtcggaatcgctagtaatcgcaggtcagcatactgcggtgaatacgttcccgggtcttgtacacaccgcccgtcacaccatgggagtgggggataccagaagtaggtagaataaccgcgaggagttcgcttaccacggtatgcttcatgactggggtg

SEQ ID NO: 3 - RNA, 1493 nt, Massiliprevotella massiliensis strain Marseille-P2439
  source 1..1493: mol_type = rRNA
agagtttgatcctggctcaggatgaacgctagctacaggcttaacacatgcaagtcgaggggaaacgatagggaaagcttgctttycytaggcgtcgaccggcgcacgggtgagtaacgcgtatccaacctgcccatgtctggggaataacccgtcgaaaggcggactaactccccatggtctccgatgaggacatctgaattggagtaaagcttcgcggacatggatggggatgcgtctgattaggtagtaggcggggtaacggcccacctagcctacgatcagtaggggttctgagaggaaggtcccccacattggaactgagacacggtccaaactcctacgggaggcagcagtgaggaatattggtcaatggacgagagtctgaaccagccaagtagcgtgcaggatgacggccctatgggttgtaaactgcttttgcgcggggataacaccctccacgtgctggaggtctgcaggtaccgcgcgaataaggaccggctaattccgtgccagcagccgcggtaatacggaaggtccgggcgttatccggatttattgggtttaaagggagcgtaggccgtgaggtaagcgtgttgtgaaatgtaggcgcccaacgtctgcactgcagcgcgaactgccccacttgagtgcgcgcaacgccggcggaactcgtcgtgtagcggtgaaatgcttagatatgacgaagaaccccgattgcgaaggcagctggcgggagcgtaactgacgctgaagctcgaaagcgcgggtatcgaacaggattagataccctggtagtccgcgcggtaaacgatggatgcccgctgtggcgcgcctggcgtgccgcggctaagcgaaagcattaagcatcccacctggggagtacgccggcaacggtgaaactcaaaggaattgacgggggcccgcacaagcggaggaacatgtggtttaattcgatgatacgcgaggaaccttacccgggcttgaactgcaggagaacgattcagagatgatgaggtccttcgggactcctgtggaggtgctgcatggttgtcgtcagctcgtgccgtgaggtgtcggcttaagtgccataacgagcgcaacccctctccgtagttgccatcgggtaatgccgggcactctgcggacactgccaccgtaaggtgtgaggaaggtggggatgacgtcaaatcagcacggcccttacgtccggggccacacacgtgttacaatggccgtcacagaggggagccgggcgaccggctcatgatccttaaaaacggtctcagttcggactggggtctgcaacccgaccccacgaagctggattcgctagtaatcgcgcatcagccatggcgcggtgaatacgttcccgggccttgtacacaccgcccgtcaagccatgaaagccgggggcgcctgaagtccgtgaccgcaaggatcggcctagggcgaaactggtgattggggctaagtcgtaacaaggtagccgt

SEQ ID NO: 4 - RNA, 1475 nt, Streptobacillus notomytis strain AHL 370-1
  source 1..1475: mol_type = rRNA
agagtttgatcctggctcaggatgaacgctgacagaatgcttaacacatgcaaatctatgttaattatgtaagcttgcttagataagagacatggtggactggtgagtaacgtgtaaagaacttacctcttagactgggataaccattagaaatgatggataatactagatattattagaagtgggcatctacttttaatgaaaggagagattgctaagagagagctttgcatcctattagctagttggtggggtaaaggcctaccaaggcgatgataggtagccggcccgagagggtgaacggccacaaggggactgagatacggcccttactcctacgggaggcagcagtggggaatattggacaatggaggaaactctgatccagcaattctgtgtgcacgaagaaggttttcggattgtaaagtgctttcagtagggaagaagaaagtgacggtacctacagaagaagcgacggctaaatacgtgccagcagccgcggtaatacgtatgtcgcaagcgttatccggaattattgggcttaaagggcatctaggcggtctaacaagttgaaggtgaaaagctgtggctcaaccatagtcttgcctacaaaactgtcagactagagtactggaaaggtgggtggaactacacgagtagaggtgaaattcgtagatatgtgtaggaatgccgatgatgaagataactcactggacagaaactgacgctgaagtgcgaaagctaggggagcaaacaggattagataccctggtagtcctagctgtaaacgatgatcactgggtgtgggggtataagcctctgtgccgaagcaaaagcgataagtgatccgcctggggagtacgtacgcaagtatgaaactcaaaggaattgacggggacccgcacaagtggtggagcatgtggtttaattcgacgcaacgcgaggaaccttaccagatcttgacatactcggaataagatggaagcatcttagtgccttcgggaaccgagatacaggtggtgcatggctgtcgacagctcgtgtcgtgagatgttgggttaagtcccgcaacgagcgaaacccctatcattagttgccatcattaagttggggactctaatgaaactgcccgcgacgagcgggaggaaggtggggatgacgtcaagtcatcatgccccttatgatctgggctacacacgtgctacaatgggtagtacaaagaggagctaagcagtgatgtggagcaaatcttaaaagctactctcagttcggattgaagtctgcaactcgacttcatgaagttggaatcactagtaatcgcaaatcagcaatgttgcggtgaatacgttctcgggtcttgtacacaccgcccgtcacaccacgagagttagttgcacctgaagttactggcctaaccgtaaggagggaagtacctaaggtgtgattagtgattggggtgaagtcgtaacaaggta

SEQ ID NO: 5 - RNA, 1533 nt, Rothia halotolerans strain YIM 90716
  source 1..1533: mol_type = rRNA
agagattagagtttgatcctggctcaggacgaacgctggcggcgtgcttaacacatgcaagtcgaacgctgaagcacccagcttgctgggtgtggatgagtggcgaacgggtgagtaatacgtgagtgaccttcccttgactctgggataagcccgggaaactgggtctaataccggatatgcactatcacctgcctgggtggtggtggaaagggttttgtactggtcttggatgggctcacggcctatcagctagttggtgaggtaatggcttaccaaggcgacgacgggtagccggcctgagagggtgaccggccacactgggactgagacacggcccagactcctacgggaggcagcagtggggaatattgcacaatgggcgcaagcctgatgcagcgacgccgcgtgagggatgacggccttcgggttgtaaacctctttcagcagggaagaagcgaaagtgacggtacctgcagaagaagcgccggctaactacgtgccagcagccgcggtaatacgtagggcgcaagcgttgtccggaattattgggcgtaaagagctcgtaggcggcttgtcgcgtctgctgtgaaagcccggggcttaaccccgtggtgtgcagtgggtacgggcaggctagagtgcagtaggggagactggaattcctggtgtagcggtgaaatgcgcagatatcaggaggaacaccgatggcgaaggcaggtctctgggctgttactgacgctgaggagcgaaagcatggggagcggacaggattagataccctggtagtccatgccgtaaacgttgggcactaggtgtgggggacattccacgttttccgcgccgtagctaacgcattaagtgccccgcctggggagtacggccgcaaggctaaaactcaaaggaattgacgggggcccgcacaagcggcggagcatgcggattaattcgatgcaacgcgaagaaccttaccaaggcttgacatacactggatcgcagcagagatgttgtttcctctttgaggctggtgtacaggtggtgcatggttgtcgtcagctcgtgtcgtgagatgttgggttaagtcccgcaacgagcgcaaccctcgttctatgttgccagcacgtgatggtggggactcataggagactgccggggtcaactcggaggaaggtggggatgacgtcaaatcatcatgccccttatgtcttgggcttcacgcatgctacaatggccggtacaatgggttgcgatactgtgaggtggagctaatcccaaaaagccggtctcagttcggattggggtctgcaactcgaccccatgaagtcggagtcgctagtaatcgcagatcagcaacgctgcggtgaatacgttcccgggccttgtacacaccgcccgtcaagtcacgaaagttggtaacacccgaagccgatggcctaacccttgtggagggagtcgtcgaaggtgggactggcgattgggactaagtcgtaacaaggtagccgtaccggaaggtgcggctggatcacctcctaa

SEQ ID NO: 6 - RNA, 1463 nt, Slackia piriformis YIT 12062
  source 1..1463: mol_type = rRNA
gatgaacgctggcggcgtgcctaacacatgcaagtcgaacggttaaggcgccttcgggcgcgcatagagtggcgaacgggtgagtaacacgtgaccaacctgccccctcctccgggacaacctcgggaaaccgaggctaataccggatggtcccgccgggccgcatggccgggcggggaaagcccaggcgggaggggatggggtcgcggcccatcaggtagtaggcggggtgacggcccacctagctgacgacgggtagccgcgctgagaggcggaccggccacattgggactgagacacggcccagactcctacgggaggcagcagtggggaattttgcgcaatgggggaaaccctgacgcagcaacgccgcgtgcgggacgaaggccttcgggtcgtaaaccgctttcagcagggaagaagaatgacggtacctgcagaagaagccccggctaactacgtgccagcagccgcggtaatacgtagggggcgagcgttatccggattcattgggcgtaaagcgcgcgtaggcgtcccttcaagcggcaccgtcgaagccgggggctcaacccccggaagcgggccgaactggggggatcgagtgcggtaggggaaggcggaattcccggtgtagcggtgaaatgcgcagatatcgggaagaacaccgacggcgaaggcagccttctgggccgccactgacgctgaggcgcgaaagctgggggagcgaacaggattagataccctggtagtcccagccgtaaacgatgggcgctaggtgtggggggagatgtccctccgtgccgcagccaacgcattaagcgccccgcctggggagtacggccgcaaggctaaaactcaaaggaattgacgggggcccgcacaagcagcggagcatgtggcttaattcgaagcaacgcgaagaaccttaccagggcttgacatcaccgtgagccgccggagacggcggggccgaaaggagcggtgacaggtggtgcatggctgtcgtcagctcgtgtcgtgagatgttgggttaagtcccgcaacgagcgcaacccccgccgcgtgttgccagcattgagttgggcactcgcgcgggactgccggcgtcaagccggaggaaggtggggacgacgtcaagtcatcatgcccctcatgccctgggctgcacacgtgctacaatggccggtacagcgggctgcgacgccgcgaggcggagcgaatcccacaaagccggccccagttcggaccgcaggctgcaacccgcctgcgcgaagccggagttgctagtaatcgcggatcagcatgccgcggtgaatacgttcccgggccttgtacacaccgcccgtcacaccacccgagtcgtctgcacccgaagccgccggccgaacccgcaaggggcggaggcgtcgaaggtgtggagggtgaggggggtgaagtcgtaacaaggtagccgtaccggaagg

SEQ ID NO: 7 - RNA, 1530 nt, Oscillibacter valericigenes strain Sjm18-20
  source 1..1530: mol_type = rRNA
tttatagagagtttgatcctggctcaggacgaacgctggcggcgtgcttaacacatgcaagtcgaacggagcacccttgattgaggtttcggccaaatgagaggaatgcttagtggcggactggtgagtaacgcgtgaggaacctgcctttcagagggggacaacagttggaaacgactgctaataccgcatgatacatttgggcgacatcgcttgaatgtcaaagatttatcgctgaaagatggcctcgcgtctgattagatagttggtgaggtaacggcccaccaagtcgacgatcagtagccggactgagaggttgaccggccacattgggactgagatacggcccagactcctacgggaggcagcagtggggaatattgggcaatggacgcaagtctgacccagcaacgccgcgtgaaggaagaaggctttcgggttgtaaacttcttttaagggggaagagtagaagacggtaccccttgaataagccacggctaactacgtgccagcagccgcggtaatacgtaggtggcaagcgttgtccggatttactgggtgtaaagggcgtgtagccgggaaggtaagtcagatgtgaaatctgggggctcaacctccaaactgcatttgaaactacttttcttgagtatcggagaggtaatcggaattccttgtgtagcggtgaaatgcgtagatataaggaagaacaccagtggcgaaggcggattactggacgacaactgacggtgaggcgcgaaagcgtggggagcaaacaggattagataccctggtagtccacgctgtaaacgatcaatactaggtgtgcggggactgaccccctgcgtgccgcagttaacacaataagtattgcacctggggagtacgatcgcaaggttgaaactcaaaggaattgacgggggcccgcacaagcggtggattatgtggtttaattcgaagcaacgcgaagaaccttaccaggacttgacatcctactaacgaggtagagatacgtcaggtgcccttcggggaaagtagagacaggtggtgcatggttgtcgtcagctcgtgtcgtgagatgttgggttaagtcccgcaacgagcgcaacccctattgttagttgctacgcaagagcactctagcgagactgccgttgacaaaacggaggaaggtggggacgacgtcaaatcatcatgccccttatgtcctgggctacacacgtaatacaatggcggtcaacagagggatgcaaagccgtgaggtggagcgaacccctaaaagccgtctcagttcggatcgcaggctgcaactcgcctgcgtgaagtcggaatcgctagtaatcgcggatcagaatgccgcggtgaatacgttcccgggccttgtacacaccgcccgtcacaccatgagagtcgggaacacccgaagtccgtagcctaacagcaatgagggcgcggccgaaggtgggtttgataattggggtgaagtcgtaacaaggtagccgtatcggaaggtgcggctggatcacctccttt

SEQ ID NO: 8 - RNA, 1485 nt, Cuneatibacter caecimuris strain BARN-424-CC-10
  source 1..1485: mol_type = rRNA
agagtttgatcctggctcaggatgaacgctggcggcgtgcttaacacatgcaagtcgaacgaagcagttgcgaggaagttttcggatggaattgcgattgactgagtggcggacgggtgagtaacgcgtgggtaacctgcctcacacagggggataacagttagaaatgactgctaataccgcataacccgctagggccgcatggcccggacggaaaagaaatatcggtgtgagatggacccgcgtctgattagctggttggtagggtaacggcctaccaaggcgacgatcagtagccgacttgagagagtgatcggccacattgggactgagacacggcccaaactcctacgggaggcagcagtggggaatattgcacaatgggggaaaccctgatgcagcgacgccgcgtgactgaagaagtacttcggtatgtaaaggtctatcagcagggaagaagaaagacggtacctgactaagaagccccggctaactacgtgccagcagccgcggtaatacgtagggggcaagcgttatccggatttactgggtgtaaagggagcgtaggcggtagcgcaagtcagaagtgaaagcccggggctcaaccccgcggactgcttttgaaactgcgtaactggagtgcaggagaggtaagtggaattcctagtgtagcggtgaaatgcgtagatattaggaggaacaccagtggcgaaggcggcttactggactgtaactgacgctgaggctcgaaagcgtggggagcaaacaggattagataccctggtagtccacgctgtaaacgatgaatactaggtgtcggggagcaaagctcttcggtgccgtcgcaaacgcagtaagtattccacctggggagtacgttcgcaagaatgaaactcaaaggaattgacggggacccgcacaagcggtggagcatgtggtttaattcgaagcaacgcgaagaaccttacctgctcttgacatccccctgacgcagaggtaatgctctgtttctttcgagacaggggagacaggtggtgcatggttgtcgtcagctcgtgtcgtgagatgttgggttaagtcccgcaacgagcgcaacccttatccttagtagccagcaggtagagctgggcactctggggagactgccggggataacccggaggaaggtggggatgacgtcaaatcatcatgccccttatgagcagggctacacacgtgctacaatggcgtaaacagagggaagcgaaggggtgacctgaagcgaatctcaaaaataacgtctcagttcggattgtagtctgcaactcgactacatgaagctggaatcgctagtaatcgcgaatcagaatgtcgcggtgaatacgttcccgggtcttgtacacaccgcccgtcacaccatgggagtcggtaacgcccgaagccagtgacctaacctgaaaagggaggagctgtcgaaggcgggactggtaactggggtgaagtcgt

SEQ ID NO: 9 - RNA, 1462 nt, Faecalibacterium prausnitzii strain ATCC 27768
  source 1..1462: mol_type = rRNA
gatcctggctcaggcgaacgctggcggcgcgcctaacacatgcaagtcgaacgagcgagagagagcttgctttctcaagcgagtggcgaacgggtgagtaacgcgtgaggaacctgcctcaaagagggggacaacagttggaaacgactgctaataccgcataagcccacgacccggcatcgggtagagggaaaaggagcaatccgctttgagatggcctcgcgtccgattagctagttggtgaggtaacggcccaccaaggcgacgatcggtagccggactgagaggttgaacggccacattgggactgagacacggcccagactcctacgggaggcagcagtggggaatattgcacaatgggggaaaccctgatgcagcgacgccgcgtggaggaagaaggtcttcggattgtaaactcctgttgttgaggaagataatgacggtactcaacaaggaagtgacggctaactacgtgccagcagccgcggtaaaacgtaggtcacaagcgttgtccggaattactgggtgtaaagggagcgcaggcgggaaggcaagttggaagtgaaatccatgggctcaacccatgaactgctttcaaaactgtttttcttgagtagtgcagaggtaggcggaattcccggtgtagcggtggaatgcgtagatatcgggaggaacaccagtggcgaaggcggcctactgggcaccaactgacgctgaggctcgaaagtgtgggtagcaaacaggattagataccctggtagtccacactgtggccgatgtttactaggtgttggaggattgaccccttcagtgccgcagttaacacaataagtaatccacctggggagtacgaccgcaaggttgaaactcaaaggaattgacgggggcccgcacaagcagtggagtatgtggtttaattcgacgcaacgcgaagaaccttaccaagtcttgacatcctgcgacgcacatagaaatatgtgtttccttcgggacgcagagacaggtggtgcatggttgtcgtcagctcgtgtcgtgagatgttgggttaagtcccgcaacgagcgcaacccttatggtcagttactacgcaagaggactctggccagactgccgttgacaaaacggaggaaggtggggatgacgtcaaatcatcatgccctttatgacttgggctacacacgtactacaatggcgttaaacaaagagaagcaagaccgcgaggtggagcaaaactcagaaacaacgtcccagttcggactgcaggctgcaactcgcctgcacgaagtcggaattgctagtaatcgcagatcagcatgctgcggtgaatacgttcccgggccttgtacacaccgcccgtcacaccatgagagccggggggacccgaagtcggtagtctaaccgcaaggaggacgccgccgaaggtaaaactggtgattggggtgaagtcgtaacaaggtac

SEQ ID NO: 10 - RNA, 1495 nt, Pseudoflavonifractor phocaeensis strain Marseille-P3064
  source 1..1495: mol_type = rRNA
agagtttgatcctggctcaggatgaacgctggcggcgtrcttaacacatgcaagtcgaacggagtgcctatgaaagaggattcgtccaattgattaggttacttagtggcggacgggtgagtaacgcgtgaggaacctgcctcggagtggggaataacaatccgaaaggattgctaataccgcatgatgcagttgggccgcatggctctgactgccaaagatttatcgctctgagatggcctcgcgtctgattagctagttggcggggtaacggcccaccaaggcgacgatcagtagccggactgagaggttgaccggccacattgggactgagacacggcccagactcctacgggaggcagcagtggggaatattgggcaatgggcgcaagcctgacccagcaacgccgcgtgaaggaagaaggctttcgggttgtaaacttcttttctcagggacgaagaaaatgacggtacctgaggaataagccacggctaactacgtgccagcagccgcggtaatacgtaggtggcaagcgttatccggatttactgggtgtaaagggcgtgtaggcgggattgcaagtcaggcgtgaaaactatgggcttaacccatagcctgcgtttgaaactgtagttcttgagtgctggagaggcaatcggaattccgtgtgtagcggtgaaatgcgtagatatacggaggaacaccagtggcgaaggcggattgctggacagtaactgacgctgaggcgcgaaagcgtggggagcaaacaggattagataccctggtagtccacgccgtaaacgatggatactaggtgtggggggtctgaccccctccgtgccgcagttaacacaataagtatcccacctggggagtacgatcgcaaggttgaaactcaaaggaattgacgggggcccgcacaagcggtggagtatgtggtttaattcgaagcaacgcgaagaaccttaccagggcttgacatccaactaacgaagcagagatgcattaggtgcccttcggggaaagttgagacaggtggtgcatggttgtcgtcagctcgtgtcgtgagatgttgggttaagtcccgcaacgagcgcaacccttattgttagttgctacgcaagagcactctagcgagactgccgttgacaaaacggaggaaggtggggacgacgtcaaatcatcatgccccttatgtcctgggccacacacgtactacaatggtggttaacagagggaggcaataccgcgaggtggagcaaatccctaaaagccatcccagttcggattgcaggctgaaacccgcctgtatgaagttggaatcgctagtaatcgcggatcagcatgccgcggtgaatacgttcccgggccttgtacacaccgcccgtcacaccatgagagtcgggaacacccgaagtccgtagcctaacagcaatgggggcgcggccgaaggtgggttcgataattggggtgaagtcgtaacaaggtagccgt

SEQ ID NO: 11 - RNA, 1477 nt, Gordonibacter urolithinfaciens strain CEBAS 1/15P
  source 1..1477: mol_type = rRNA
tgctcaggatgaacgctggcggcgtgcctaacacatgcaagtcgaacgattaaggcgccttcgggcgcgaatagagtggcgaacgggtgagtaacacgtgaccaacctgcccccctccccgggataacgcgaggaaacccgcgctaataccggatactccgcccctcccgcatgggaggggcgggaaagccccgacggagggggatggggtcgcggcccattaggtagacggcggggcaacggcccaccgtgcctgcgatgggtagccgggttgagagaccgaccggccacattgggactgagatacggcccagactcctacgggaggcagcagtggggaattttgcgcaatggggggaaccctgacgcagcaacgccgcgtgcgggacgaaggccttcgggttgtaaaccgctttcagcagggaagaagttgacggtacctgcagaagaagccccggctaactacgtgccagcagccgcggtaatacgtagggggcgagcgttatccggattcattgggcgtaaagcgcgcgtaggcggcccgtcaagcggaacctctaacccgagggctcaacccccggccgggttccgaactggcaggctcgagtctggtagaggaagatggaattcccggtgtagcggtggaatgcgcagatatcgggaagaacaccgatggcgaaggcagtcttctgggccgcgactgacgctgaggcgcgaaagctgggggagcgaacaggattagataccctggtagtcccagccgtaaacgatgggcgctaggtgtggggggatcatccctccgtgccgcagccaacgcattaagcgccccgcctggggagtacggccgcaaggctaaaactcaaaggaattgacgggggcccgcacaagcagcggagcatgtggcttaattcgaagcaacgcgaagaaccttaccagggcttgacatgctggtgaagccggggaaacccggtggccgagaggagccagcgcaggtggtgcatggctgtcgtcagctcgtgtcgtgagatgttgggttaagtcccgcaacgagcgcaacccctgccatatgttgccagcattcagttggggactcatatgggactgccggcgtcaagccggaggaaggtggggacgacgtcaagtcatcatgccctttatgccctgggctgcacacgtgctacaatggccggtacaacgggccgcgacctggcgacaggaagcgaatccctcaaagccggccccagttcggatcggaggctgcaacccgcctccgtgaagtcggagttgctagtaatcgcggatcagcatgccgcggtgaatacgttcccgggccttgtacacaccgcccgtcacaccacccgagtcgtctgcacccgaagccgccggccgaacccgcaaggggcggaggcgtcgaaggtgtggagggtaaggggggtgaagtcgtaacaaggtagccgtaccggaaggtgcggctgga

SEQ ID NO: 12 - RNA, 1463 nt, Neisseria wadsworthii 9715 strain WC 05-9715
  source 1..1463: mol_type = rRNA
attgaacgctggcggcatgctttacacatgcaagtcgaacggcagcgggggagagcttgctttcctgccggcgagtggcgaacgggtgagtaatgcatcggaacgtaccgagtagtgggggataactgtccgaaaggatggctaataccgcatacgctttgcgaaggaaagcgggggctcttaggacctcgcgctattcgagcggccgatgtctgattagctagttggtggggtaaaggcctaccaaggcgacgatcagtagcgggtctgagaggatgatccgccacactgggactgagacacggcccagactcctacgggaggcagcagtggggaattttggacaatggggggaaccctgatccagccatgccgcgtgtctgaagaaggccttcgggttgtaaaggacttttgtcagggaagaaaagcttcgggttaataccctggagtgatgacggtacctgaagaataagcaccggctaactacgtgccagcagccgcggtaatacgtagggtgcgagcgttaatcggaattactgggcgtaaagcgagcgcagacggttacttaagcaggatgtgaaatccccgggctcaacctgggaactgcgttctgaactgggtgactagagtatgtcagaggggggtagaattccacgtgtagcagtgaaatgcgtagagatgtggaggaataccgatggcgaaggcagccccctgggataatactgacgttcatgctcgaaagcgtgggtagcaaacaggattagataccctggtagtccacgccctaaacgatgtcaattagctgttggggcacttgatgctttagtagcgtagctaacgcgtgaaattgaccgcctggggagtacggtcgcaagattaaaactcaaaggaattgacggggacccgcacaagcggtggatgatgtggattaattcgatgcaacgcgaagaaccttacctggtcttgacatgtacggaatcctccggagacggaggagtgccttcgggagccgtaacacaggtgctgcatggctgtcgtcagctcgtgtcgtgagatgttgggttaagtcccgcaacgagcgcaacccttgtcattagttgccatcatttagttgggcactctaatgagactgccggtgacaaaccggaggaaggtggggatgacgtcaagtcctcatggcccttatgaccagggcttcacacgtcatacaatggtcggtacagagggtagccaagccgcgaggtggagccaatcccacaaaaccgatcgtagtccggattgcactctgcaactcgagtgcatgaagtcggaatcgctagtaatcgcaggtcagcatactgcggtgaatacgttcccgggtcttgtacacaccgcccgtcacaccatgggagtgggggataccagaagtaggtagggtaaccgcaaggagcccgcttaccacggtatgcttcatgactggggtg

SEQ ID NO: 13 - RNA, 1506 nt, Fusobacterium gastrosuis strain CDW1
  source 1..1506: mol_type = rRNA
tgaacgaagagtttgatcctggctcaggatgaacgctgacagaatgcttaacacatgcaagtctacttgaacttcggtttgggtggcggacgggtgagtaacgcgtaaagaacttgcctcacagactgggacaacatttggaaacgaatgctaataccggatattatgagatatgcgcatgcataacttatgaaagctatatgcgctgtgagagagctttgcgtcccattagctagttggagaggtaacggctcaccaaggcgatgatgggtagccggcctgagagggtgaacggccacaaggggactgagacacggcccttactcctacgggaggcagcagtggggaatattggacaatggaccaagagtctgatccagcaattctgtgtgcacgatgaagtttttcggaatgtaaagtgctttcagttgggaagaagaaagtgacggtaccaacagaagaagcgacggctaaatacgtgccagcagccgcggtaatacgtatgtcgcaagcgttatccggatttattgggcgtaaagcgcgtctaggcggcatagtaagtctgatgtgaaaatgcggggctcaactccgtattgcgttggaaactgctatgctagagtactggagaggtaagcggaactacaagtgtagaggtgaaattcgtagatatttgtaggaatgccgatggggaagccagcttactggacagatactgacgctaaagcgcgaaagcgtgggtagcaaacaggattagataccctggtagtccacgccgtaaacgatgattactaggtgttgggggtcgaacctcagcgcccaagctaacgcgataagtaatccgcctggggagtacgtacgcaagtatgaaactcaaaggaattgacggggacccgcacaagcggtggagcatgtggtttaattcgacgcaacgcgaggaaccttaccagcgtttgacatcctaagaagtctatagagatatggatgtgctccttcgggagaacttagtgacaggtggtgcatggctgtcgtcagctcgtgtcgtgagatgttgggttaagtcccgcaacgagcgcaacccctttcgtatgttaccatcattaagttggggactcatgcgatactgcctgcgatgagcaggaggaaggtggggatgacgtcaagtcatcatgccccttatacgctgggctacacacgtgctacaatgggtagtacagagagaagcgaaactgcgaggtggagcaaatctcagaaaactattcttagttcggattgtactctgcaactcgagtacatgaagttggaatcgctagtaatcgcaaatcagctatgttgcggtgaatacgttctcgggtcttgtacacaccgcccgtcacaccacgagagttggttgcacctgaagtaacaggcctaaccgtaaggagggatgttccgagggtgtgattagcgattggggtgaagtcgtaacaaggtatccgtacgggaacgtgcggatggatcacctccttt

SEQ ID NO: 14 - RNA, 1547 nt, Lactococcus allomyrinae strain 1JSPR-7
  source 1..1547: mol_type = rRNA
ttatttgagagtttgatcctggctcaggacgaacgctggcggcgtgcctaatacatgcaagttgagcgctgaaggaaggtacttgtaccgactggaagagcagcgaacgggtgagtaacgcgtggggaatctgcctttgagcgggggacaacatttggaaacgaatgctaataccgcataacaactttaaacacaagttaaaagtttgaaagatgcaaaagcatcactcagagatgatcccgcgttgtattagctagttggtgaggtaaaggctcaccaaggcgatgatacatagccgacctgagagggtgatcggccacattgggactgagacacggcccaaactcctacgggaggcagcagtagggaatcttcggcaatggacgaaagtctgaccgagcaacgccgcgtgagtgaagaaggttttcggatcgtaaaactctgttgttagagaagaacgtgtgtgggagtggaaaatccatgcagtgacggtatctaaccagaaagggacggctaactacgtgccagcagccgcggtaatacgtaggtcccgagcgttgtccggatttattgggcgtaaagcgagcgcaggtggtttattaagtctggtgtaaaaggcagtggctcaaccattgtatgcattggaaactggtagacttgagtgcaggagaggagagtggaattccatgtgtagcggtgaaatgcgtagatatatggaggaacaccggtggcgaaagcggctctctggcctgtaactgacactgaggctcgaaagcgtggggagcaaacaggattagataccctggtagtccacgccgtaaacgatgagtgctagatgtaggaagctataagttttctgtatcgcagctaacgcaataagcactccgcctggggagtacgaccgcaaggttgaaactcaaaggaattgacgggggcccgcacaagcggtggagcatgtggtttaattcgaagcaacgcgaagaaccttaccaggtcttgacatcccgatgctatccttagagataaggagttacttcggtacatcggtgacaggtggtgcatggttgtcgtcagctcgtgtcgtgagatgttgggttaagtcccgcaacgagcgcaacccctattactagttgccatcattaagttgggcactctagtgagactgccggtgataaaccggaggaaggtggggatgacgtcaaatcatcatgccccttatgacctgggctacacacgtgctacaatggatggtacaacgagtcgcgagacagtgatgtttagctaatctcttaaaaccattctcagttcggattgtaggctgcaactcgcctacatgaagtcggaatcgctagtaatcgcggatcagcacgccgcggtgaatacgttcccgggccttgtacacaccgcccgtcacaccacgggagttgggagtacccgaagtaggttgcctaaccgcaaggagggcgcttcctaaggtaagaccgatgactggggtgaagtcgtaacaaggtagccgtatcggaaggtgcggctggatcacctccttt

SEQ ID NO: 15 - RNA, 1563 nt, Lactobacillus mulieris strain c10Ua161M
  source 1..1563: mol_type = rRNA
caaaatgagagtttgatcctggctcaggacgaacgctggcggcgtgcctaatacatgcaagtcgagcgagcttgcctattgaaattcttcggaatggacatagatacaagctagcggcggatgggtgagtaacgcgtgggtaacctgcccttaagtctgggataccatttggaaacagatgctaataccggataaaagctactttcgcatgaaagaagtttaaaaggcggcgtaagctgtcgctaaaggatggacctgcgatgcattagctagttggtaaggtaacggcttaccaaggcgatgatgcatagccgagttgagagactgatcggccacattgggactgagacacggcccaaactcctacgggaggcagcagtagggaatcttccacaatggacgcaagtctgatggagcaacgccgcgtgagtgaagaaggttttcggatcgtaaagctctgttgttggtgaagaaggatagaggtagtaactggcctttatttgacggtaatcaaccagaaagtcacggctaactacgtgccagcagccgcggtaatacgtaggtggcaagcgttgtccggatttattgggcgtaaagcgagcgcaggcggattgataagtctgatgtgaaagccttcggctcaaccgaagaactgcatcagaaactgtcaatcttgagtgcagaagaggagagtggaactccatgtgtagcggtggaatgcgtagatatatggaagaacaccagtggcgaaggcggctctctggtctgtaactgacgctgaggctcgaaagcatgggtagcgaacaggattagataccctggtagtccatgccgtaaacgatgagtgctaagtgttgggaggtttccgcctctcagtgctgcagctaacgcattaagcactccgcctggggagtacgaccgcaaggttgaaactcaaaggaattgacgggggcccgcacaagcggtggagcatgtggtttaattcgaagcaacgcgaagaaccttaccaggtcttgacatcctttgaccacctaagagattaggttttcccttcggggacaaagagacaggtggtgcatggctgtcgtcagctcgtgtcgtgagatgttgggttaagtcccgcaacgagcgcaacccttgttaatagttgccagcattaagttgggcactctattgagactgccggtgacaaaccggaggaaggtggggatgacgtcaagtcatcatgccccttatgacctgggctacacacgtgctacaatgggcagtacaacgagaagcgaacctgtgaaggcaagcggatctcttaaagctgttctcagttcggactgtaggctgcaactcgcctacacgaagctggaatcgctagtaatcgcggatcagcacgccgcggtgaatacgttcccgggccttgtacacaccgcccgtcacaccatgagagtttgtaacacccaaagtcggtgaggtaacctttggagccagccgcctaaggtgggacagatgattagggtgaagtcgtaacaaggtagccgtaggagaacctgcggctggatcacctccttt